European Patent Application EP 4 144 364 A1, published March 8, 2023. Title: 一种治疗脊髓性肌萎缩症的方法和药物. Applicant: 泰伦基国际有限公司. The sequence listing filed with the application follows.

SEQUENCE LISTING (18 sequences)

SEQ ID NO: 1 - DNA, 2376 bp, 人工序列
  不含有信号肽的天然纤溶酶原(Glu-PLG，Glu-纤维蛋白溶酶原)核酸序列
gagcctctggatgactatgtgaatacccagggggcttcactgttcagtgtcactaagaagcagctgggagcaggaagtatagaagaatgtgcagcaaaatgtgaggaggacgaagaattcacctgcagggcattccaatatcacagtaaagagcaacaatgtgtgataatggctgaaaacaggaagtcctccataatcattaggatgagagatgtagttttatttgaaaagaaagtgtatctctcagagtgcaagactgggaatggaaagaactacagagggacgatgtccaaaacaaaaaatggcatcacctgtcaaaaatggagttccacttctccccacagacctagattctcacctgctacacacccctcagagggactggaggagaactactgcaggaatccagacaacgatccgcaggggccctggtgctatactactgatccagaaaagagatatgactactgcgacattcttgagtgtgaagaggaatgtatgcattgcagtggagaaaactatgacggcaaaatttccaagaccatgtctggactggaatgccaggcctgggactctcagagcccacacgctcatggatacattccttccaaatttccaaacaagaacctgaagaagaattactgtcgtaaccccgatagggagctgcggccttggtgtttcaccaccgaccccaacaagcgctgggaactttgtgacatcccccgctgcacaacacctccaccatcttctggtcccacctaccagtgtctgaagggaacaggtgaaaactatcgcgggaatgtggctgttaccgtgtccgggcacacctgtcagcactggagtgcacagacccctcacacacataacaggacaccagaaaacttcccctgcaaaaatttggatgaaaactactgccgcaatcctgacggaaaaagggccccatggtgccatacaaccaacagccaagtgcggtgggagtactgtaagataccgtcctgtgactcctccccagtatccacggaacaattggctcccacagcaccacctgagctaacccctgtggtccaggactgctaccatggtgatggacagagctaccgaggcacatcctccaccaccaccacaggaaagaagtgtcagtcttggtcatctatgacaccacaccggcaccagaagaccccagaaaactacccaaatgctggcctgacaatgaactactgcaggaatccagatgccgataaaggcccctggtgttttaccacagaccccagcgtcaggtgggagtactgcaacctgaaaaaatgctcaggaacagaagcgagtgttgtagcacctccgcctgttgtcctgcttccagatgtagagactccttccgaagaagactgtatgtttgggaatgggaaaggataccgaggcaagagggcgaccactgttactgggacgccatgccaggactgggctgcccaggagccccatagacacagcattttcactccagagacaaatccacgggcgggtctggaaaaaaattactgccgtaaccctgatggtgatgtaggtggtccctggtgctacacgacaaatccaagaaaactttacgactactgtgatgtccctcagtgtgcggccccttcatttgattgtgggaagcctcaagtggagccgaagaaatgtcctggaagggttgtaggggggtgtgtggcccacccacattcctggccctggcaagtcagtcttagaacaaggtttggaatgcacttctgtggaggcaccttgatatccccagagtgggtgttgactgctgcccactgcttggagaagtccccaaggccttcatcctacaaggtcatcctgggtgcacaccaagaagtgaatctcgaaccgcatgttcaggaaatagaagtgtctaggctgttcttggagcccacacgaaaagatattgccttgctaaagctaagcagtcctgccgtcatcactgacaaagtaatcccagcttgtctgccatccccaaattatgtggtcgctgaccggaccgaatgtttcatcactggctggggagaaacccaaggtacttttggagctggccttctcaaggaagcccagctccctgtgattgagaataaagtgtgcaatcgctatgagtttctgaatggaagagtccaatccaccgaactctgtgctgggcatttggccggaggcactgacagttgccagggtgacagtggaggtcctctggtttgcttcgagaaggacaaatacattttacaaggagtcacttcttggggtcttggctgtgcacgccccaataagcctggtgtctatgttcgtgtttcaaggtttgttacttggattgagggagtgatgagaaataattaa

SEQ ID NO: 2 - protein, 791 aa, 人工序列
  不含有信号肽的天然纤溶酶原(Glu-PLG，Glu-纤维蛋白溶酶原)氨基酸序列
EPLDDYVNTQGASLFSVTKKQLGAGSIEECAAKCEEDEEFTCRAFQYHSKEQQCVIMAENRKSSIIIRMRDVVLFEKKVYLSECKTGNGKNYRGTMSKTKNGITCQKWSSTSPHRPRFSPATHPSEGLEENYCRNPDNDPQGPWCYTTDPEKRYDYCDILECEEECMHCSGENYDGKISKTMSGLECQAWDSQSPHAHGYIPSKFPNKNLKKNYCRNPDRELRPWCFTTDPNKRWELCDIPRCTTPPPSSGPTYQCLKGTGENYRGNVAVTVSGHTCQHWSAQTPHTHNRTPENFPCKNLDENYCRNPDGKRAPWCHTTNSQVRWEYCKIPSCDSSPVSTEQLAPTAPPELTPVVQDCYHGDGQSYRGTSSTTTTGKKCQSWSSMTPHRHQKTPENYPNAGLTMNYCRNPDADKGPWCFTTDPSVRWEYCNLKKCSGTEASVVAPPPVVLLPDVETPSEEDCMFGNGKGYRGKRATTVTGTPCQDWAAQEPHRHSIFTPETNPRAGLEKNYCRNPDGDVGGPWCYTTNPRKLYDYCDVPQCAAPSFDCGKPQVEPKKCPGRVVGGCVAHPHSWPWQVSLRTRFGMHFCGGTLISPEWVLTAAHCLEKSPRPSSYKVILGAHQEVNLEPHVQEIEVSRLFLEPTRKDIALLKLSSPAVITDKVIPACLPSPNYVVADRTECFITGWGETQGTFGAGLLKEAQLPVIENKVCNRYEFLNGRVQSTELCAGHLAGGTDSCQGDSGGPLVCFEKDKYILQGVTSWGLGCARPNKPGVYVRVSRFVTWIEGVMRNN

SEQ ID NO: 3 - DNA, 2433 bp, 人工序列
  含有信号肽的天然纤溶酶原(来源于swiss prot)的核酸序列
atggaacataaggaagtggttcttctacttcttttatttctgaaatcaggtcaaggagagcctctggatgactatgtgaatacccagggggcttcactgttcagtgtcactaagaagcagctgggagcaggaagtatagaagaatgtgcagcaaaatgtgaggaggacgaagaattcacctgcagggcattccaatatcacagtaaagagcaacaatgtgtgataatggctgaaaacaggaagtcctccataatcattaggatgagagatgtagttttatttgaaaagaaagtgtatctctcagagtgcaagactgggaatggaaagaactacagagggacgatgtccaaaacaaaaaatggcatcacctgtcaaaaatggagttccacttctccccacagacctagattctcacctgctacacacccctcagagggactggaggagaactactgcaggaatccagacaacgatccgcaggggccctggtgctatactactgatccagaaaagagatatgactactgcgacattcttgagtgtgaagaggaatgtatgcattgcagtggagaaaactatgacggcaaaatttccaagaccatgtctggactggaatgccaggcctgggactctcagagcccacacgctcatggatacattccttccaaatttccaaacaagaacctgaagaagaattactgtcgtaaccccgatagggagctgcggccttggtgtttcaccaccgaccccaacaagcgctgggaactttgtgacatcccccgctgcacaacacctccaccatcttctggtcccacctaccagtgtctgaagggaacaggtgaaaactatcgcgggaatgtggctgttaccgtgtccgggcacacctgtcagcactggagtgcacagacccctcacacacataacaggacaccagaaaacttcccctgcaaaaatttggatgaaaactactgccgcaatcctgacggaaaaagggccccatggtgccatacaaccaacagccaagtgcggtgggagtactgtaagataccgtcctgtgactcctccccagtatccacggaacaattggctcccacagcaccacctgagctaacccctgtggtccaggactgctaccatggtgatggacagagctaccgaggcacatcctccaccaccaccacaggaaagaagtgtcagtcttggtcatctatgacaccacaccggcaccagaagaccccagaaaactacccaaatgctggcctgacaatgaactactgcaggaatccagatgccgataaaggcccctggtgttttaccacagaccccagcgtcaggtgggagtactgcaacctgaaaaaatgctcaggaacagaagcgagtgttgtagcacctccgcctgttgtcctgcttccagatgtagagactccttccgaagaagactgtatgtttgggaatgggaaaggataccgaggcaagagggcgaccactgttactgggacgccatgccaggactgggctgcccaggagccccatagacacagcattttcactccagagacaaatccacgggcgggtctggaaaaaaattactgccgtaaccctgatggtgatgtaggtggtccctggtgctacacgacaaatccaagaaaactttacgactactgtgatgtccctcagtgtgcggccccttcatttgattgtgggaagcctcaagtggagccgaagaaatgtcctggaagggttgtaggggggtgtgtggcccacccacattcctggccctggcaagtcagtcttagaacaaggtttggaatgcacttctgtggaggcaccttgatatccccagagtgggtgttgactgctgcccactgcttggagaagtccccaaggccttcatcctacaaggtcatcctgggtgcacaccaagaagtgaatctcgaaccgcatgttcaggaaatagaagtgtctaggctgttcttggagcccacacgaaaagatattgccttgctaaagctaagcagtcctgccgtcatcactgacaaagtaatcccagcttgtctgccatccccaaattatgtggtcgctgaccggaccgaatgtttcatcactggctggggagaaacccaaggtacttttggagctggccttctcaaggaagcccagctccctgtgattgagaataaagtgtgcaatcgctatgagtttctgaatggaagagtccaatccaccgaactctgtgctgggcatttggccggaggcactgacagttgccagggtgacagtggaggtcctctggtttgcttcgagaaggacaaatacattttacaaggagtcacttcttggggtcttggctgtgcacgccccaataagcctggtgtctatgttcgtgtttcaaggtttgttacttggattgagggagtgatgagaaataattaa

SEQ ID NO: 4 - protein, 810 aa, 人工序列
  含有信号肽的天然纤溶酶原(来源于swiss prot)的氨基酸序列
MEHKEVVLLLLLFLKSGQGEPLDDYVNTQGASLFSVTKKQLGAGSIEECAAKCEEDEEFTCRAFQYHSKEQQCVIMAENRKSSIIIRMRDVVLFEKKVYLSECKTGNGKNYRGTMSKTKNGITCQKWSSTSPHRPRFSPATHPSEGLEENYCRNPDNDPQGPWCYTTDPEKRYDYCDILECEEECMHCSGENYDGKISKTMSGLECQAWDSQSPHAHGYIPSKFPNKNLKKNYCRNPDRELRPWCFTTDPNKRWELCDIPRCTTPPPSSGPTYQCLKGTGENYRGNVAVTVSGHTCQHWSAQTPHTHNRTPENFPCKNLDENYCRNPDGKRAPWCHTTNSQVRWEYCKIPSCDSSPVSTEQLAPTAPPELTPVVQDCYHGDGQSYRGTSSTTTTGKKCQSWSSMTPHRHQKTPENYPNAGLTMNYCRNPDADKGPWCFTTDPSVRWEYCNLKKCSGTEASVVAPPPVVLLPDVETPSEEDCMFGNGKGYRGKRATTVTGTPCQDWAAQEPHRHSIFTPETNPRAGLEKNYCRNPDGDVGGPWCYTTNPRKLYDYCDVPQCAAPSFDCGKPQVEPKKCPGRVVGGCVAHPHSWPWQVSLRTRFGMHFCGGTLISPEWVLTAAHCLEKSPRPSSYKVILGAHQEVNLEPHVQEIEVSRLFLEPTRKDIALLKLSSPAVITDKVIPACLPSPNYVVADRTECFITGWGETQGTFGAGLLKEAQLPVIENKVCNRYEFLNGRVQSTELCAGHLAGGTDSCQGDSGGPLVCFEKDKYILQGVTSWGLGCARPNKPGVYVRVSRFVTWIEGVMRNN

SEQ ID NO: 5 - DNA, 2145 bp, 人工序列
  LYS77-PLG(Lys-纤溶酶原)核酸序列
aaagtgtatctctcagagtgcaagactgggaatggaaagaactacagagggacgatgtccaaaacaaaaaatggcatcacctgtcaaaaatggagttccacttctccccacagacctagattctcacctgctacacacccctcagagggactggaggagaactactgcaggaatccagacaacgatccgcaggggccctggtgctatactactgatccagaaaagagatatgactactgcgacattcttgagtgtgaagaggaatgtatgcattgcagtggagaaaactatgacggcaaaatttccaagaccatgtctggactggaatgccaggcctgggactctcagagcccacacgctcatggatacattccttccaaatttccaaacaagaacctgaagaagaattactgtcgtaaccccgatagggagctgcggccttggtgtttcaccaccgaccccaacaagcgctgggaactttgtgacatcccccgctgcacaacacctccaccatcttctggtcccacctaccagtgtctgaagggaacaggtgaaaactatcgcgggaatgtggctgttaccgtgtccgggcacacctgtcagcactggagtgcacagacccctcacacacataacaggacaccagaaaacttcccctgcaaaaatttggatgaaaactactgccgcaatcctgacggaaaaagggccccatggtgccatacaaccaacagccaagtgcggtgggagtactgtaagataccgtcctgtgactcctccccagtatccacggaacaattggctcccacagcaccacctgagctaacccctgtggtccaggactgctaccatggtgatggacagagctaccgaggcacatcctccaccaccaccacaggaaagaagtgtcagtcttggtcatctatgacaccacaccggcaccagaagaccccagaaaactacccaaatgctggcctgacaatgaactactgcaggaatccagatgccgataaaggcccctggtgttttaccacagaccccagcgtcaggtgggagtactgcaacctgaaaaaatgctcaggaacagaagcgagtgttgtagcacctccgcctgttgtcctgcttccagatgtagagactccttccgaagaagactgtatgtttgggaatgggaaaggataccgaggcaagagggcgaccactgttactgggacgccatgccaggactgggctgcccaggagccccatagacacagcattttcactccagagacaaatccacgggcgggtctggaaaaaaattactgccgtaaccctgatggtgatgtaggtggtccctggtgctacacgacaaatccaagaaaactttacgactactgtgatgtccctcagtgtgcggccccttcatttgattgtgggaagcctcaagtggagccgaagaaatgtcctggaagggttgtaggggggtgtgtggcccacccacattcctggccctggcaagtcagtcttagaacaaggtttggaatgcacttctgtggaggcaccttgatatccccagagtgggtgttgactgctgcccactgcttggagaagtccccaaggccttcatcctacaaggtcatcctgggtgcacaccaagaagtgaatctcgaaccgcatgttcaggaaatagaagtgtctaggctgttcttggagcccacacgaaaagatattgccttgctaaagctaagcagtcctgccgtcatcactgacaaagtaatcccagcttgtctgccatccccaaattatgtggtcgctgaccggaccgaatgtttcatcactggctggggagaaacccaaggtacttttggagctggccttctcaaggaagcccagctccctgtgattgagaataaagtgtgcaatcgctatgagtttctgaatggaagagtccaatccaccgaactctgtgctgggcatttggccggaggcactgacagttgccagggtgacagtggaggtcctctggtttgcttcgagaaggacaaatacattttacaaggagtcacttcttggggtcttggctgtgcacgccccaataagcctggtgtctatgttcgtgtttcaaggtttgttacttggattgagggagtgatgagaaataattaa

SEQ ID NO: 6 - protein, 714 aa, 人工序列
  LYS77-PLG(Lys-纤溶酶原)氨基酸序列
KVYLSECKTGNGKNYRGTMSKTKNGITCQKWSSTSPHRPRFSPATHPSEGLEENYCRNPDNDPQGPWCYTTDPEKRYDYCDILECEEECMHCSGENYDGKISKTMSGLECQAWDSQSPHAHGYIPSKFPNKNLKKNYCRNPDRELRPWCFTTDPNKRWELCDIPRCTTPPPSSGPTYQCLKGTGENYRGNVAVTVSGHTCQHWSAQTPHTHNRTPENFPCKNLDENYCRNPDGKRAPWCHTTNSQVRWEYCKIPSCDSSPVSTEQLAPTAPPELTPVVQDCYHGDGQSYRGTSSTTTTGKKCQSWSSMTPHRHQKTPENYPNAGLTMNYCRNPDADKGPWCFTTDPSVRWEYCNLKKCSGTEASVVAPPPVVLLPDVETPSEEDCMFGNGKGYRGKRATTVTGTPCQDWAAQEPHRHSIFTPETNPRAGLEKNYCRNPDGDVGGPWCYTTNPRKLYDYCDVPQCAAPSFDCGKPQVEPKKCPGRVVGGCVAHPHSWPWQVSLRTRFGMHFCGGTLISPEWVLTAAHCLEKSPRPSSYKVILGAHQEVNLEPHVQEIEVSRLFLEPTRKDIALLKLSSPAVITDKVIPACLPSPNYVVADRTECFITGWGETQGTFGAGLLKEAQLPVIENKVCNRYEFLNGRVQSTELCAGHLAGGTDSCQGDSGGPLVCFEKDKYILQGVTSWGLGCARPNKPGVYVRVSRFVTWIEGVMRNN

SEQ ID NO: 7 - DNA, 1245 bp, 人工序列
  delta-plg(delta-纤溶酶原)核酸序列
gagcctctggatgactatgtgaatacccagggggcttcactgttcagtgtcactaagaagcagctgggagcaggaagtatagaagaatgtgcagcaaaatgtgaggaggacgaagaattcacctgcagggcattccaatatcacagtaaagagcaacaatgtgtgataatggctgaaaacaggaagtcctccataatcattaggatgagagatgtagttttatttgaaaagaaagtgtatctctcagagtgcaagactgggaatggaaagaactacagagggacgatgtccaaaacaaaaaatggcatcacctgtcaaaaatggagttccacttctccccacagacctagattctcacctgctacacacccctcagagggactggaggagaactactgcaggaatccagacaacgatccgcaggggccctggtgctatactactgatccagaaaagagatatgactactgcgacattcttgagtgtgaagaggcggccccttcatttgattgtgggaagcctcaagtggagccgaagaaatgtcctggaagggttgtaggggggtgtgtggcccacccacattcctggccctggcaagtcagtcttagaacaaggtttggaatgcacttctgtggaggcaccttgatatccccagagtgggtgttgactgctgcccactgcttggagaagtccccaaggccttcatcctacaaggtcatcctgggtgcacaccaagaagtgaatctcgaaccgcatgttcaggaaatagaagtgtctaggctgttcttggagcccacacgaaaagatattgccttgctaaagctaagcagtcctgccgtcatcactgacaaagtaatcccagcttgtctgccatccccaaattatgtggtcgctgaccggaccgaatgtttcatcactggctggggagaaacccaaggtacttttggagctggccttctcaaggaagcccagctccctgtgattgagaataaagtgtgcaatcgctatgagtttctgaatggaagagtccaatccaccgaactctgtgctgggcatttggccggaggcactgacagttgccagggtgacagtggaggtcctctggtttgcttcgagaaggacaaatacattttacaaggagtcacttcttggggtcttggctgtgcacgccccaataagcctggtgtctatgttcgtgtttcaaggtttgttacttggattgagggagtgatgagaaataattaa

SEQ ID NO: 8 - protein, 414 aa, 人工序列
  delta-plg(delta-纤溶酶原)氨基酸序列
EPLDDYVNTQGASLFSVTKKQLGAGSIEECAAKCEEDEEFTCRAFQYHSKEQQCVIMAENRKSSIIIRMRDVVLFEKKVYLSECKTGNGKNYRGTMSKTKNGITCQKWSSTSPHRPRFSPATHPSEGLEENYCRNPDNDPQGPWCYTTDPEKRYDYCDILECEEAAPSFDCGKPQVEPKKCPGRVVGGCVAHPHSWPWQVSLRTRFGMHFCGGTLISPEWVLTAAHCLEKSPRPSSYKVILGAHQEVNLEPHVQEIEVSRLFLEPTRKDIALLKLSSPAVITDKVIPACLPSPNYVVADRTECFITGWGETQGTFGAGLLKEAQLPVIENKVCNRYEFLNGRVQSTELCAGHLAGGTDSCQGDSGGPLVCFEKDKYILQGVTSWGLGCARPNKPGVYVRVSRFVTWIEGVMRNN

SEQ ID NO: 9 - DNA, 1104 bp, 人工序列
  Mini-plg(小纤维蛋白溶酶原)核酸序列
gtcaggtgggagtactgcaacctgaaaaaatgctcaggaacagaagcgagtgttgtagcacctccgcctgttgtcctgcttccagatgtagagactccttccgaagaagactgtatgtttgggaatgggaaaggataccgaggcaagagggcgaccactgttactgggacgccatgccaggactgggctgcccaggagccccatagacacagcattttcactccagagacaaatccacgggcgggtctggaaaaaaattactgccgtaaccctgatggtgatgtaggtggtccctggtgctacacgacaaatccaagaaaactttacgactactgtgatgtccctcagtgtgcggccccttcatttgattgtgggaagcctcaagtggagccgaagaaatgtcctggaagggttgtaggggggtgtgtggcccacccacattcctggccctggcaagtcagtcttagaacaaggtttggaatgcacttctgtggaggcaccttgatatccccagagtgggtgttgactgctgcccactgcttggagaagtccccaaggccttcatcctacaaggtcatcctgggtgcacaccaagaagtgaatctcgaaccgcatgttcaggaaatagaagtgtctaggctgttcttggagcccacacgaaaagatattgccttgctaaagctaagcagtcctgccgtcatcactgacaaagtaatcccagcttgtctgccatccccaaattatgtggtcgctgaccggaccgaatgtttcatcactggctggggagaaacccaaggtacttttggagctggccttctcaaggaagcccagctccctgtgattgagaataaagtgtgcaatcgctatgagtttctgaatggaagagtccaatccaccgaactctgtgctgggcatttggccggaggcactgacagttgccagggtgacagtggaggtcctctggtttgcttcgagaaggacaaatacattttacaaggagtcacttcttggggtcttggctgtgcacgccccaataagcctggtgtctatgttcgtgtttcaaggtttgttacttggattgagggagtgatgagaaataattaa

SEQ ID NO: 10 - protein, 367 aa, 人工序列
  Mini-plg(小纤维蛋白溶酶原)氨基酸序列
VRWEYCNLKKCSGTEASVVAPPPVVLLPDVETPSEEDCMFGNGKGYRGKRATTVTGTPCQDWAAQEPHRHSIFTPETNPRAGLEKNYCRNPDGDVGGPWCYTTNPRKLYDYCDVPQCAAPSFDCGKPQVEPKKCPGRVVGGCVAHPHSWPWQVSLRTRFGMHFCGGTLISPEWVLTAAHCLEKSPRPSSYKVILGAHQEVNLEPHVQEIEVSRLFLEPTRKDIALLKLSSPAVITDKVIPACLPSPNYVVADRTECFITGWGETQGTFGAGLLKEAQLPVIENKVCNRYEFLNGRVQSTELCAGHLAGGTDSCQGDSGGPLVCFEKDKYILQGVTSWGLGCARPNKPGVYVRVSRFVTWIEGVMRNN

SEQ ID NO: 11 - DNA, 750 bp, 人工序列
  Micro-plg(微纤维蛋白溶酶原)核酸序列
gccccttcatttgattgtgggaagcctcaagtggagccgaagaaatgtcctggaagggttgtaggggggtgtgtggcccacccacattcctggccctggcaagtcagtcttagaacaaggtttggaatgcacttctgtggaggcaccttgatatccccagagtgggtgttgactgctgcccactgcttggagaagtccccaaggccttcatcctacaaggtcatcctgggtgcacaccaagaagtgaatctcgaaccgcatgttcaggaaatagaagtgtctaggctgttcttggagcccacacgaaaagatattgccttgctaaagctaagcagtcctgccgtcatcactgacaaagtaatcccagcttgtctgccatccccaaattatgtggtcgctgaccggaccgaatgtttcatcactggctggggagaaacccaaggtacttttggagctggccttctcaaggaagcccagctccctgtgattgagaataaagtgtgcaatcgctatgagtttctgaatggaagagtccaatccaccgaactctgtgctgggcatttggccggaggcactgacagttgccagggtgacagtggaggtcctctggtttgcttcgagaaggacaaatacattttacaaggagtcacttcttggggtcttggctgtgcacgccccaataagcctggtgtctatgttcgtgtttcaaggtttgttacttggattgagggagtgatgagaaataattaa

SEQ ID NO: 12 - protein, 249 aa, 人工序列
  Micro-plg(微纤维蛋白溶酶原)氨基酸序列
APSFDCGKPQVEPKKCPGRVVGGCVAHPHSWPWQVSLRTRFGMHFCGGTLISPEWVLTAAHCLEKSPRPSSYKVILGAHQEVNLEPHVQEIEVSRLFLEPTRKDIALLKLSSPAVITDKVIPACLPSPNYVVADRTECFITGWGETQGTFGAGLLKEAQLPVIENKVCNRYEFLNGRVQSTELCAGHLAGGTDSCQGDSGGPLVCFEKDKYILQGVTSWGLGCARPNKPGVYVRVSRFVTWIEGVMRNN

SEQ ID NO: 13 - DNA, 684 bp, 人工序列
  丝氨酸蛋白酶(结构)域的核酸序列
gttgtaggggggtgtgtggcccacccacattcctggccctggcaagtcagtcttagaacaaggtttggaatgcacttctgtggaggcaccttgatatccccagagtgggtgttgactgctgcccactgcttggagaagtccccaaggccttcatcctacaaggtcatcctgggtgcacaccaagaagtgaatctcgaaccgcatgttcaggaaatagaagtgtctaggctgttcttggagcccacacgaaaagatattgccttgctaaagctaagcagtcctgccgtcatcactgacaaagtaatcccagcttgtctgccatccccaaattatgtggtcgctgaccggaccgaatgtttcatcactggctggggagaaacccaaggtacttttggagctggccttctcaaggaagcccagctccctgtgattgagaataaagtgtgcaatcgctatgagtttctgaatggaagagtccaatccaccgaactctgtgctgggcatttggccggaggcactgacagttgccagggtgacagtggaggtcctctggtttgcttcgagaaggacaaatacattttacaaggagtcacttcttggggtcttggctgtgcacgccccaataagcctggtgtctatgttcgtgtttcaaggtttgttacttggattgagggagtgatgaga

SEQ ID NO: 14 - protein, 228 aa, 人工序列
  丝氨酸蛋白酶(结构)域的氨基酸序列
VVGGCVAHPHSWPWQVSLRTRFGMHFCGGTLISPEWVLTAAHCLEKSPRPSSYKVILGAHQEVNLEPHVQEIEVSRLFLEPTRKDIALLKLSSPAVITDKVIPACLPSPNYVVADRTECFITGWGETQGTFGAGLLKEAQLPVIENKVCNRYEFLNGRVQSTELCAGHLAGGTDSCQGDSGGPLVCFEKDKYILQGVTSWGLGCARPNKPGVYVRVSRFVTWIEGVMR

SEQ ID NO: 15 - DNA, 20 bp, 人工序列
  引物
gcggcggcagtggtggcggc

SEQ ID NO: 16 - DNA, 22 bp, 人工序列
  引物
agtagatcggacagattttgct

SEQ ID NO: 17 - DNA, 24 bp, 人工序列
  引物
gctgatgctttgggaagtatgtta

SEQ ID NO: 18 - DNA, 20 bp, 人工序列
  引物
attccagatctgtctgatcg